European Patent Specification EP 3 448 879 B1, published February 26, 2025. Title: Peptides. Applicant: Immunocore Limited Adaptimmune Limited. The sequence listing filed with the application follows.

SEQUENCE LISTING (17 sequences)

SEQ ID NO: 1 - protein, 11 aa, Homo sapiens
SLLALPQDLQA

SEQ ID NO: 2 - protein, 9 aa, Homo sapiens
VLTSGIVFV

SEQ ID NO: 3 - protein, 9 aa, Homo sapiens
TLIPVCWTA

SEQ ID NO: 4 - protein, 15 aa, Homo sapiens
AISRGPSEYPTKNYV

SEQ ID NO: 5 - protein, 9 aa, Homo sapiens
GLLLLGGGL

SEQ ID NO: 6 - protein, 113 aa, Homo sapiens
KQEVTQIPAALSVPEGENLVLNCSFTDSAIYNLQWFRQDPGKGLTSLLLIQSSQREQTSGRLNASLDKSSGRSTLYIAASQPGDSATYLCAVRHLSNDYKLSFGAGTTVTVRA

SEQ ID NO: 7 - protein, 114 aa, Homo sapiens
NAGVTQTPKFQVLKTGQSMTLQCAQDMNHEYMSWYRQDPGMGLRLIHYSVGAGITDQGEVPNGYNVSRSTTEDFPLRLLSAAPSQTSVYFCASKRGFDEGSPLHFGNGTRLTVT

SEQ ID NO: 8 - protein, 112 aa, Homo sapiens
KQEVTQIPAALSVPEGENLVLNCSFTDSAIYNLQWFRQDPGKGLTSLLLIQSSQREQTSGRLNASLDKSSGRSTLYIAASQPGDSATYLCAVRHNQGGKLIFGQGTELSVKP

SEQ ID NO: 9 - protein, 112 aa, Homo sapiens
NAGVTQTPKFRVLKTGQSMTLLCAQDMNHEYMYWYRQDPGMGLRLIHYSVGAGITDQGEVPNGYNVSRLNKREFSLRLESAAPSQTSVYFCASSDRGVYEQYFGPGTRLTVT

SEQ ID NO: 10 - protein, 114 aa, Homo sapiens
KQEVTQIPAALSVPEGENLVLNCSFTDSAIYNLQWFRQDPGKGLTSLLLIQSSQREQTSGRLNASLDKSSGRSTLYIAASQPGDSATYLCAVRPLGGGYQKVTFGTGTKLQVIP

SEQ ID NO: 11 - protein, 115 aa, Homo sapiens
NAGVTQTPKFRVLKTGQSMTLQCAQDMNHNSMYWYRQDPGMGLRLIYYSASEGTTDKGEVPNGYNVSRLNKREFSLRLESAAPSQTSVYFCASSDTGTSVTGELFFGEGSRLTVL

SEQ ID NO: 12 - protein, 111 aa, Homo sapiens
KQEVTQIPAALSVPEGENLVLNCSFTDSAIYNLQWFRQDPGKGLTSLLLIQSSQREQTSGRLNASLDKSSGRSTLYIAASQPGDSATYLCAVQGYGTALIFGKGTTLSVSS

SEQ ID NO: 13 - protein, 114 aa, Homo sapiens
NAGVTQTPKFQVLKTGQSMTLQCAQDMNHEYMSWYRQDPGMGLRLIHYSVGAGITDQGEVPNGYNVSRSTTEDFPLRLLSAAPSQTSVYFCASSQGPYMNTEAFFGQGTRLTVV

SEQ ID NO: 14 - protein, 111 aa, Homo sapiens
KQEVTQIPAALSVPEGENLVLNCSFTDSAIYNLQWFRQDPGKGLTSLLLIQSSQREQTSGRLNASLDKSSGRSTLYIAASQPGDSATYLCAAKAAGNKLTFGGGTRVLVKP

SEQ ID NO: 15 - protein, 114 aa, Homo sapiens
NAGVTQTPKFQVLKTGQSMTLQCAQDMNHNSMYWYRQDPGMGLRLIYYSASEGTTDKGEVPNGYNVSRLNKREFSLRLESAAPSQTSVYFCASSESLGVTGTAFFGQGTRLTVV

SEQ ID NO: 16 - protein, 112 aa, Homo sapiens
KQEVTQIPAALSVPEGENLVLNCSFTDSAIYNLQWFRQDPGKGLTSLLLIQSSQREQTSGRLNASLDKSSGRSTLYIAASQPGDSATYLCAVKKDAGNKLTFGGGTRVLVKP

SEQ ID NO: 17 - protein, 114 aa, Homo sapiens
NAGVTQTPKFQVLKTGQSMTLQCAQDMNHNSMYWYRQDPGMGLRLIYYSASEGTTDKGEVPNGYNVSRLNKREFPLRLLSAAPSQTSVYFCASSRRLGASSEAFFGQGTRLTVV